European Patent Application EP 4 729 529 A1, published April 22, 2026. Title: 白介素-23受体的肽抑制剂制备及其用途. Applicant: 西藏海思科制药有限公司. Application CN. The sequence listing filed with the application follows.

SEQUENCE LISTING (3 sequences)

SEQ ID NO: 1 - protein, 13 aa, synthetic construct
  MOD_RES 1: note = X is (Ac)Xa1, Xa1 is independently selected from Pen, Pcn, Asn, Ala, Ala (3-amino), Ala (2-ethene), Ala (3-azido), Ala (2-ethene), Val (2-ethene), 2,4-DIAMINO-BUTYRIC ACID, Ser, Cys, Hcys, Glu.
  MOD_RES 2: note = X is selected from Asn, His or analogues of Asn and His.
  MOD_RES 4: note = X is selected from Trp or its analogues.
  MOD_RES 5: note = Lysine is acetylated.
  MOD_RES 6: note = X is independently selected from Pen, Pcn, Asn, Ala, Ala (3-amino), Ala (2-ethene), Ala (3-azido), Ala (2-ethene), Val (2-ethene), 2,4-DIAMINO-BUTYRIC ACID, Ser, Cys, Hcys, Glu.
  MOD_RES 7: note = X is selected from Phe or its analogues.
  MOD_RES 8: note = X is selected from Phe, Trp, 2-Nal or analogues of Phe, Trp and 2-Nal.
  MOD_RES 9: note = X is selected from Thp or its analogues.
  MOD_RES 12: note = X is 3-Pal.
  MOD_RES 13: note = X is Sarc(NH2).
XXTXKXXXXENXX

SEQ ID NO: 2 - protein, 13 aa, synthetic construct
  MOD_RES 1: note = X is (Ac)Xa1, Xa1 is independently selected from Pen, Pcn, Asn, Ala, Ala (3-amino), Ala (2-ethene), Ala (3-azido), Ala (2-ethene), Val (2-ethene), 2,4-DIAMINO-BUTYRIC ACID, Ser, Cys, Hcys, Glu.
  MOD_RES 2: note = X is selected from Asn, His or analogues of Asn and His.
  MOD_RES 4: note = Tryptophan is methylated.
  MOD_RES 5: note = Lysine is acetylated.
  MOD_RES 6: note = X is independently selected from Pen, Pcn, Asn, Ala, Ala (3-amino), Ala (2-ethene), Ala (3-azido), Ala (2-ethene), Val (2-ethene), 2,4-DIAMINO-BUTYRIC ACID, Ser, Cys, Hcys, Glu.
  MOD_RES 7: note = X is selected from Phe or its analogues.
  MOD_RES 8: note = X is selected from Phe, Trp, 2-Nal or analogues of Phe, Trp and 2-Nal.
  MOD_RES 9: note = X is selected from Thp or its analogues.
  MOD_RES 12: note = X is 3-Pal.
  MOD_RES 13: note = X is Sarc(NH2).
XXTWKXXXXENXX

SEQ ID NO: 3 - protein, 13 aa, synthetic construct
  MOD_RES 1: note = X is independently selected from Pen, Pcn, Asn, Ala, Ala (3-amino), Ala (2-ethene), Ala (3-azido), Ala (2-ethene), Val (2-ethene), 2,4-DIAMINO-BUTYRIC ACID, Ser, Cys, Hcys, Glu.
  MOD_RES 4: note = Tryptophan is methylated.
  MOD_RES 5: note = Lysine is acetylated.
  MOD_RES 6: note = X is independently selected from Pen, Pcn, Asn, Ala, Ala (3-amino), Ala (2-ethene), Ala (3-azido), Ala (2-ethene), Val (2-ethene), 2,4-DIAMINO-BUTYRIC ACID, Ser, Cys, Hcys, Glu.
  MOD_RES 7: note = X is selected from Phe or its analogues.
  MOD_RES 8: note = X is 2-Nal.
  MOD_RES 9: note = X is selected from Thp or its analogues.
  MOD_RES 11: note = X is selected from Asn, Lys or analogues of Asn and Lys.
  MOD_RES 12: note = X is selected from 3-Pal, Phe, Asp or analogues of 3-Pal, Phe and Asp.
  MOD_RES 13: note = X is Sarc.
XNTWKXXXXEXXX